European Patent Specification EP 3 452 515 B1, published August 20, 2025. Title: HER-2 binding antibodies. Applicant: MAB DISCOVERY GMBH. The sequence listing filed with the application follows.

SEQUENCE LISTING (104 sequences)

SEQ ID NO: 1 - protein, 116 aa, Artificial Sequence
  recombinant chimeric antibody
QSLEESGGRLVTPGTPLTLTCTVSGFSLSSYNMGWVRQAPGKGLEWIGIISHSDNTYYASWAKGRFTISKTSTTVDLKMTSPTTEDTATYFCARGAAGGSGAYNLWGQGMLVTVSS

SEQ ID NO: 2 - protein, 116 aa, Artificial Sequence
  recombinant chimeric antibody
QSVEESGGRLVTPGTPLTLTCTVSGFSLSNYNMAWVRQAPGEGLEYIGIINAGGTAYYASWAKGRITISKTSTTVDLKISSPTAEDTATYFCARSYTSNSGAFNIWGPGTLVTVSS

SEQ ID NO: 3 - protein, 114 aa, Artificial Sequence
  recombinant chimeric antibody
QSVEESGGRLVTPGTPLTLTCTVSGFSLSSYAMSWVRQAPGKGLEWIGIIYSGGNAHYASWAKGRFTISRTSTTVDLKMTSLTTEDTATYFCARGDDSSGLRLWGQGTLVTVSS

SEQ ID NO: 4 - protein, 116 aa, Artificial Sequence
  recombinant chimeric antibody
QSVEESGGRLVTPGTPLTLTCTVSGFSLSNYGVSWVRQAPGKGLEYIGIISGSGFTYYASWAKGRFTISKTSTTVDLKITSPTTKDTATYFCARGVVPGYNAGGLWGQGTLVTVSS

SEQ ID NO: 5 - protein, 120 aa, Artificial Sequence
  recombinant chimeric antibody
QSVEESGGRLVTPGTPLTLTCTVSGFSLSSYAMSWVRQAPGKGLEWIGIIYAISDNTWFASWAKGRFTISKTSTTVDLKITSPTTEDTATYFCARALYAGYTAGYYFSLWGPGTLVTVSS

SEQ ID NO: 6 - protein, 120 aa, Artificial Sequence
  recombinant chimeric antibody
QSLEESGGDLVKPGASLTLTCTASGFSFSSSYYMCWLRQAPGKGLEWVACIYGGSSSSTYYASWAKGRFTISKTSSTTVTLQMTSLTAADTATYFCARDQIYDDSGFNLWGPGTLVTVSS

SEQ ID NO: 7 - protein, 110 aa, Artificial Sequence
  recombinant chimeric antibody
DIVMTQTPASVEAAVGGTVTIKCQASQSISTALGWYQQKPGQRPKLLIYGASNLEFGVPSRFKGSGSGTEYTLTISDLESGDAATYYCQCSAYGSRYVGGFGGGTEVVVK

SEQ ID NO: 8 - protein, 110 aa, Artificial Sequence
  recombinant chimeric antibody
DVVMTQTPASVSEPVGGTVTIKCQASQSIGNALAWYQQKPGQPPKLLIYGASNLESGVSSRFRGSRSGTEFTLTISDLESADAATYYCQCSAYGSVYVGTFGGGTEVVVK

SEQ ID NO: 9 - protein, 110 aa, Artificial Sequence
  recombinant chimeric antibody
DVVMTQTPASVSEPVGGTVTIKCQASQSISNLLAWYQQKPGQRPKLLMSYASSLASGVSSRFKGSRSGTEYTLTISDLECADAATYYCQCTDVGSNYLGAFGGGTEVVVK

SEQ ID NO: 10 - protein, 110 aa, Artificial Sequence
  recombinant chimeric antibody
DIVMTQTPASVSEPVGGTVTIKCQASQGISTALAWYQQKPGQRPKLLIYSASTLASGVSSRFKGSGSGTQFTLTISDLECADAATYYCQCTAAGSVSVGAFGGGTEVVVN

SEQ ID NO: 11 - protein, 112 aa, Artificial Sequence
  recombinant chimeric antibody
DPVLTQTPSSASEPVGGTVTIKCQASQSIYSYLSWYQQKPGQPPELLIYSASTLASGVPSRFKGSGSGTQFTLTISDLECADSATYYCQNNNGGSYSSAFGAFGGGTEVVVK

SEQ ID NO: 12 - protein, 112 aa, Artificial Sequence
  recombinant chimeric antibody
DIVMTQTPSSVSEPVGGTVTIKCQASQSISIYLSWYQQKPGQPPKRLIYKASTLESGVPSRFKGSGSGTEFTLTISDLECADAATYYCQSNYGSGSSSWEGAFGGGTEVVVK

SEQ ID NO: 13 - protein, 5 aa, Artificial Sequence
  recombinant chimeric antibody
SYNMG

SEQ ID NO: 14 - protein, 5 aa, Artificial Sequence
  recombinant chimeric antibody
NYNMA

SEQ ID NO: 15 - protein, 5 aa, Artificial Sequence
  recombinant chimeric antibody
SYAMS

SEQ ID NO: 16 - protein, 5 aa, Artificial Sequence
  recombinant chimeric antibody
NYGVS

SEQ ID NO: 17 - protein, 5 aa, Artificial Sequence
  recombinant chimeric antibody
SYAMS

SEQ ID NO: 18 - protein, 6 aa, Artificial Sequence
  recombinant chimeric antibody
SSYYMC

SEQ ID NO: 19 - protein, 16 aa, Artificial Sequence
  recombinant chimeric antibody
IISHSDNTYYASWAKG

SEQ ID NO: 20 - protein, 16 aa, Artificial Sequence
  recombinant chimeric antibody
IINAGGTAYYASWAKG

SEQ ID NO: 21 - protein, 16 aa, Artificial Sequence
  recombinant chimeric antibody
IIYSGGNAHYASWAKG

SEQ ID NO: 22 - protein, 16 aa, Artificial Sequence
  recombinant chimeric antibody
IISGSGFTYYASWAKG

SEQ ID NO: 23 - protein, 17 aa, Artificial Sequence
  recombinant chimeric antibody
IIYAISDNTWFASWAKG

SEQ ID NO: 24 - protein, 18 aa, Artificial Sequence
  recombinant chimeric antibody
CIYGGSSSSTYYASWAKG

SEQ ID NO: 25 - protein, 11 aa, Artificial Sequence
  recombinant chimeric antibody
GAAGGSGAYNL

SEQ ID NO: 26 - protein, 11 aa, Artificial Sequence
  recombinant chimeric antibody
SYTSNSGAFNI

SEQ ID NO: 27 - protein, 9 aa, Artificial Sequence
  recombinant chimeric antibody
GDDSSGLRL

SEQ ID NO: 28 - protein, 11 aa, Artificial Sequence
  recombinant chimeric antibody
GVVPGYNAGGL

SEQ ID NO: 29 - protein, 14 aa, Artificial Sequence
  recombinant chimeric antibody
ALYAGYTAGYYFSL

SEQ ID NO: 30 - protein, 11 aa, Artificial Sequence
  recombinant chimeric antibody
DQIYDDSGFNL

SEQ ID NO: 31 - protein, 11 aa, Artificial Sequence
  recombinant chimeric antibody
QASQSISTALG

SEQ ID NO: 32 - protein, 11 aa, Artificial Sequence
  recombinant chimeric antibody
QASQSIGNALA

SEQ ID NO: 33 - protein, 11 aa, Artificial Sequence
  recombinant chimeric antibody
QASQSISNLLA

SEQ ID NO: 34 - protein, 11 aa, Artificial Sequence
  recombinant chimeric antibody
QASQGISTALA

SEQ ID NO: 35 - protein, 11 aa, Artificial Sequence
  recombinant chimeric antibody
QASQSIYSYLS

SEQ ID NO: 36 - protein, 11 aa, Artificial Sequence
  recombinant chimeric antibody
QASQSISIYLS

SEQ ID NO: 37 - protein, 7 aa, Artificial Sequence
  recombinant chimeric antibody
GASNLEF

SEQ ID NO: 38 - protein, 7 aa, Artificial Sequence
  recombinant chimeric antibody
GASNLES

SEQ ID NO: 39 - protein, 7 aa, Artificial Sequence
  recombinant chimeric antibody
YASSLAS

SEQ ID NO: 40 - protein, 7 aa, Artificial Sequence
  recombinant chimeric antibody
SASTLAS

SEQ ID NO: 41 - protein, 7 aa, Artificial Sequence
  recombinant chimeric antibody
SASTLAS

SEQ ID NO: 42 - protein, 7 aa, Artificial Sequence
  recombinant chimeric antibody
KASTLES

SEQ ID NO: 43 - protein, 12 aa, Artificial Sequence
  recombinant chimeric antibody
QCSAYGSRYVGG

SEQ ID NO: 44 - protein, 12 aa, Artificial Sequence
  recombinant chimeric antibody
QCSAYGSVYVGT

SEQ ID NO: 45 - protein, 12 aa, Artificial Sequence
  recombinant chimeric antibody
QCTDVGSNYLGA

SEQ ID NO: 46 - protein, 12 aa, Artificial Sequence
  recombinant chimeric antibody
QCTAAGSVSVGA

SEQ ID NO: 47 - protein, 14 aa, Artificial Sequence
  recombinant chimeric antibody
QNNNGGSYSSAFGA

SEQ ID NO: 48 - protein, 14 aa, Artificial Sequence
  recombinant chimeric antibody
QSNYGSGSSSWEGA

SEQ ID NO: 49 - protein, 29 aa, Artificial Sequence
  recombinant chimeric antibody
QSLEESGGRLVTPGTPLTLTCTVSGFSLS

SEQ ID NO: 50 - protein, 29 aa, Artificial Sequence
  recombinant chimeric antibody
QSVEESGGRLVTPGTPLTLTCTVSGFSLS

SEQ ID NO: 51 - protein, 29 aa, Artificial Sequence
  recombinant chimeric antibody
QSVEESGGRLVTPGTPLTLTCTVSGFSLS

SEQ ID NO: 52 - protein, 29 aa, Artificial Sequence
  recombinant chimeric antibody
QSVEESGGRLVTPGTPLTLTCTVSGFSLS

SEQ ID NO: 53 - protein, 29 aa, Artificial Sequence
  recombinant chimeric antibody
QSVEESGGRLVTPGTPLTLTCTVSGFSLS

SEQ ID NO: 54 - protein, 29 aa, Artificial Sequence
  recombinant chimeric antibody
QSLEESGGDLVKPGASLTLTCTASGFSFS

SEQ ID NO: 55 - protein, 14 aa, Artificial Sequence
  recombinant chimeric antibody
WVRQAPGKGLEWIG

SEQ ID NO: 56 - protein, 14 aa, Artificial Sequence
  recombinant chimeric antibody
WVRQAPGEGLEYIG

SEQ ID NO: 57 - protein, 14 aa, Artificial Sequence
  recombinant chimeric antibody
WVRQAPGKGLEWIG

SEQ ID NO: 58 - protein, 14 aa, Artificial Sequence
  recombinant chimeric antibody
WVRQAPGKGLEYIG

SEQ ID NO: 59 - protein, 14 aa, Artificial Sequence
  recombinant chimeric antibody
WVRQAPGKGLEWIG

SEQ ID NO: 60 - protein, 14 aa, Artificial Sequence
  recombinant chimeric antibody
WLRQAPGKGLEWVA

SEQ ID NO: 61 - protein, 30 aa, Artificial Sequence
  recombinant chimeric antibody
RFTISKTSTTVDLKMTSPTTEDTATYFCAR

SEQ ID NO: 62 - protein, 30 aa, Artificial Sequence
  recombinant chimeric antibody
RITISKTSTTVDLKISSPTAEDTATYFCAR

SEQ ID NO: 63 - protein, 30 aa, Artificial Sequence
  recombinant chimeric antibody
RFTISRTSTTVDLKMTSLTTEDTATYFCAR

SEQ ID NO: 64 - protein, 30 aa, Artificial Sequence
  recombinant chimeric antibody
RFTISKTSTTVDLKITSPTTKDTATYFCAR

SEQ ID NO: 65 - protein, 30 aa, Artificial Sequence
  recombinant chimeric antibody
RFTISKTSTTVDLKITSPTTEDTATYFCAR

SEQ ID NO: 66 - protein, 31 aa, Artificial Sequence
  recombinant chimeric antibody
RFTISKTSSTTVTLQMTSLTAADTATYFCAR

SEQ ID NO: 67 - protein, 11 aa, Artificial Sequence
  recombinant chimeric antibody
WGQGMLVTVSS

SEQ ID NO: 68 - protein, 11 aa, Artificial Sequence
  recombinant chimeric antibody
WGPGTLVTVSS

SEQ ID NO: 69 - protein, 11 aa, Artificial Sequence
  recombinant chimeric antibody
WGQGTLVTVSS

SEQ ID NO: 70 - protein, 11 aa, Artificial Sequence
  recombinant chimeric antibody
WGQGTLVTVSS

SEQ ID NO: 71 - protein, 11 aa, Artificial Sequence
  recombinant chimeric antibody
WGPGTLVTVSS

SEQ ID NO: 72 - protein, 11 aa, Artificial Sequence
  recombinant chimeric antibody
WGPGTLVTVSS

SEQ ID NO: 73 - protein, 23 aa, Artificial Sequence
  recombinant chimeric antibody
DIVMTQTPASVEAAVGGTVTIKC

SEQ ID NO: 74 - protein, 23 aa, Artificial Sequence
  recombinant chimeric antibody
DVVMTQTPASVSEPVGGTVTIKC

SEQ ID NO: 75 - protein, 23 aa, Artificial Sequence
  recombinant chimeric antibody
DVVMTQTPASVSEPVGGTVTIKC

SEQ ID NO: 76 - protein, 23 aa, Artificial Sequence
  recombinant chimeric antibody
DIVMTQTPASVSEPVGGTVTIKC

SEQ ID NO: 77 - protein, 23 aa, Artificial Sequence
  recombinant chimeric antibody
DPVLTQTPSSASEPVGGTVTIKC

SEQ ID NO: 78 - protein, 23 aa, Artificial Sequence
  recombinant chimeric antibody
DIVMTQTPSSVSEPVGGTVTIKC

SEQ ID NO: 79 - protein, 15 aa, Artificial Sequence
  recombinant chimeric antibody
WYQQKPGQRPKLLIY

SEQ ID NO: 80 - protein, 15 aa, Artificial Sequence
  recombinant chimeric antibody
WYQQKPGQPPKLLIY

SEQ ID NO: 81 - protein, 15 aa, Artificial Sequence
  recombinant chimeric antibody
WYQQKPGQRPKLLMS

SEQ ID NO: 82 - protein, 15 aa, Artificial Sequence
  recombinant chimeric antibody
WYQQKPGQRPKLLIY

SEQ ID NO: 83 - protein, 15 aa, Artificial Sequence
  recombinant chimeric antibody
WYQQKPGQPPELLIY

SEQ ID NO: 84 - protein, 15 aa, Artificial Sequence
  recombinant chimeric antibody
WYQQKPGQPPKRLIY

SEQ ID NO: 85 - protein, 32 aa, Artificial Sequence
  recombinant chimeric antibody
GVPSRFKGSGSGTEYTLTISDLESGDAATYYC

SEQ ID NO: 86 - protein, 32 aa, Artificial Sequence
  recombinant chimeric antibody
GVSSRFRGSRSGTEFTLTISDLESADAATYYC

SEQ ID NO: 87 - protein, 32 aa, Artificial Sequence
  recombinant chimeric antibody
GVSSRFKGSRSGTEYTLTISDLECADAATYYC

SEQ ID NO: 88 - protein, 32 aa, Artificial Sequence
  recombinant chimeric antibody
GVSSRFKGSGSGTQFTLTISDLECADAATYYC

SEQ ID NO: 89 - protein, 32 aa, Artificial Sequence
  recombinant chimeric antibody
GVPSRFKGSGSGTQFTLTISDLECADSATYYC

SEQ ID NO: 90 - protein, 32 aa, Artificial Sequence
  recombinant chimeric antibody
GVPSRFKGSGSGTEFTLTISDLECADAATYYC

SEQ ID NO: 91 - protein, 10 aa, Artificial Sequence
  recombinant chimeric antibody
FGGGTEVVVK

SEQ ID NO: 92 - protein, 10 aa, Artificial Sequence
  recombinant chimeric antibody
FGGGTEVVVK

SEQ ID NO: 93 - protein, 10 aa, Artificial Sequence
  recombinant chimeric antibody
FGGGTEVVVK

SEQ ID NO: 94 - protein, 10 aa, Artificial Sequence
  recombinant chimeric antibody
FGGGTEVVVN

SEQ ID NO: 95 - protein, 10 aa, Artificial Sequence
  recombinant chimeric antibody
FGGGTEVVVK

SEQ ID NO: 96 - protein, 10 aa, Artificial Sequence
  recombinant chimeric antibody
FGGGTEVVVK

SEQ ID NO: 97 - protein, 107 aa, Homo sapiens [sequence omitted]

SEQ ID NO: 98 - protein, 329 aa, Homo sapiens
ASTKGPSVFPLAPSSKSTSGGTAALGCLVKDYFPEPVTVSWNSGALTSGVHTFPAVLQSSGLYSLSSVVTVPSSSLGTQTYICNVNHKPSNTKVDKKVEPKSCDKTHTCPPCPAPELLGGPSVFLFPPKPKDTLMISRTPEVTCVVVDVSHEDPEVKFNWYVDGVEVHNAKTKPREEQYNSTYRVVSVLTVLHQDWLNGKEYKCKVSNKALPAPIEKTISKAKGQPREPQVYTLPPSREEMTKNQVSLTCLVKGFYPSDIAVEWESNGQPENNYKTTPPVLDSDGSFFLYSKLTVDKSRWQQGNVFSCSVMHEALHNHYTQKSLSLSPG

SEQ ID NO: 99 - protein, 331 aa, Homo sapiens
ASTKGPSVFPLAPSSKSTSGGTAALGCLVKDYFPEPVTVSWNSGALTSGVHTFPAVLQSSGLYSLSSVVTVPSSSLGTQTYICNVNHKPSNTKVDKKVEPPKSCDKTHTCPPCPAPELLGGPSVFLFPPKPKDTLMISRTPEVTCVVVDVSHEDPEVKFNWYVDGVEVHNAKTKPREEQYNSTYRVVSVLTVLHQDWLNGKEYKCKVSNKALPAPIEKTISKAKGQPREPQVYTLPPSRDELTKNQVSLTCLVKGFYPSDIAVEWESNGQPENNYKTTPPVLDSDGSFFLYSKLTVDKSRWQQGNVFSCSVMHEALHNHYTQKSLSLSPGK

SEQ ID NO: 100 - protein, 119 aa, Artificial Sequence
  humanized VR
QVQLEESGGRVVQPGTSLRLSCAASGFSLSNYGVSWVRQAPGKGLEYVAIISGSGFTYYASWAKGRFTISKDTSKNTVVMQMTSLRAEDTATYFCARGVVPGYNAGGLWGQGTLVTVSS

SEQ ID NO: 101 - protein, 119 aa, Artificial Sequence
  humanized VR
EEHLEESGGRLVKPGTSLRLSCTVSGFSLSNYGVSWVRQAPGRGLEYVSIISGSGFTYYASWAKGRFTISKDTARDSVYLQMNSLRAEDTATYFCARGVVPGYNAGGLWGQGTLVTVSS

SEQ ID NO: 102 - protein, 110 aa, Artificial Sequence
  humanized VR
DIQMTQSPSSLSASVGDRITITCQASQGISTALAWYQQKPGQVPKLLIYSASTLASGVPSRFKGSGSGTEFTLTISSLQAEDVATYYCQCTAAGSVSVGAFGGGTEVVIK

SEQ ID NO: 103 - protein, 110 aa, Artificial Sequence
  humanized VR
DIVMTQSPSSVSASVGDRVTITCQASQGISTALAWYQQKPGQAPKLLIYSASTLASGVPSRFKGSGSGTDFTLTISSLQPEDSATYYCQCTAAGSVSVGAFGQGTELVIK

SEQ ID NO: 104 - protein, 110 aa, Artificial Sequence
  humanized VR
DIELTQSPSSVSASVGDRVTITCQASQGISTALAWYQQKPGQAPKLLIYSASTLASGVPSRFKGSGSGTDFTLTISSLQSEDSATYYCQCTAAGSVSVGAFGGGTKVVIE